European Patent Specification EP 3 565 585 B1, published November 13, 2024. Title: THERAPEUTIC METHOD. Applicant: Apitope International NV. The sequence listing filed with the application follows.

SEQUENCE LISTING (6 sequences)

SEQ ID NO: 1 - protein, 15 aa, Artificial Sequence
  Synthetic peptide
PRHRDTGILDSIGRF

SEQ ID NO: 2 - protein, 17 aa, Artificial sequence
  Synthetic peptide
ENPVVHFFKNIVTPRTP

SEQ ID NO: 3 - protein, 15 aa, Artificial sequence
  Synthetic peptide
ASDYKSAHKGFKGVD

SEQ ID NO: 4 - protein, 15 aa, Artificial sequence
  Synthetic peptide
GFKGVDAQGTLSKIF

SEQ ID NO: 5 - protein, 21 aa, Artificial sequence
  Synthetic peptide
KKKKYVSIDVTLQQLESHKKK

SEQ ID NO: 6 - protein, 15 aa, Artificial sequence
  Synthetic peptide
GLKMFPDLTKVYSTD